European Patent Specification EP 3 516 080 B1, published November 5, 2025. Title: Constructs for Continuous Monitoring of Live Cells. Applicant: The Broad Institute Blainey, Paul Borrajo, Jacob Najia, Mohamad Kulshreshtha, Ankur Dixit, Atray. The sequence listing filed with the application follows.

SEQUENCE LISTING (12 sequences)

SEQ ID NO: 1 - DNA, 1590 bp, Artificial Sequence
  MLV gag
atgggccagactgttaccactcccttaagtttgaccttaggtcactggaaagatgtcgagcggatcgctcacaaccagtcggtagatgtcaagaagagacgttgggttaccttctgctctgcagaatggccaacctttaacgtcggatggccgcgagacggcacctttaaccgagacctcatcacccaggttaagatcaaggtcttttcacctggcccgcatggacacccagaccaggtcccctacatcgtgacctgggaagccttggcttttgacccccctccctgggtcaagccctttgtacaccctaagcctccgcctcctcttcctccatccgccccgtctctcccccttgaacctcctcgttcgaccccgcctcgatcctccctttatccagccctcactccttctctaggcgccaaacctaaacctcaagttctttctgacagtggggggccgctcatcgacctacttacagaagaccccccgccttatagggacccaagaccacccccttccgacagggacggaaatggtggagaagcgacccctgcgggagaggcaccggacccctccccaatggcatctcgcctacgtgggagacgggagccccctgtggccgactccactacctcgcaggcattccccctccgcgcaggaggaaacggacagcttcaatactggccgttctcctcttctgacctttacaactggaaaaataataacccttctttttctgaagatccaggtaaactgacagctctgatcgagtctgttctcatcacccatcagcccacctgggacgactgtcagcagctgttggggactctgctgaccggagaagaaaaacaacgggtgctcttagaggctagaaaggcggtgcggggcgatgatgggcgccccactcaactgcccaatgaagtcgatgccgcttttcccctcgagcgcccagactgggattacaccacccaggcaggtaggaaccacctagtccactatcgccagttgctcctagcgggtctccaaaacgcgggcagaagccccaccaatttggccaaggtaaaaggaataacacaagggcccaatgagtctccctcggccttcctagagagacttaaggaagcctatcgcaggtacactccttatgaccctgaggacccagggcaagaaactaatgtgtctatgtctttcatttggcagtctgccccagacattgggagaaagttagagaggttagaagatttaaaaaacaagacgcttggagatttggttagagaggcagaaaagatctttaataaacgagaaaccccggaagaaagagaggaacgtatcaggagagaaacagaggaaaaagaagaacgccgtaggacagaggatgagcagaaagagaaagaaagagatcgtaggagacatagagagatgagcaagctattggccactgtcgttagtggacagaaacaggatagacagggaggagaacgaaggaggtcccaactcgatcgcgaccagtgtgcctactgcaaagaaaaggggcactgggctaaagattgtcccaagaaaccacgaggacctcggggaccaagaccgcag

SEQ ID NO: 2 - DNA, 1935 bp, Artificial Sequence
  PABPC4 - RNA binding protein fragment
atgaacgctgcggccagcagctaccccatggcctccctgtacgtgggcgacctgcattcggacgtcaccgaggccatgctgtacgaaaagttcagccccgcggggcctgtgctgtccatccgggtctgccgcgatatgatcacccgccgctccctgggctatgcctacgtcaacttccagcagccggccgacgctgagcgggctttggacaccatgaactttgatgtgattaagggaaagccaatccgcatcatgtggtctcagagggatccctctttgagaaaatctggtgtgggaaacgtcttcatcaagaacctggacaaatctatagataacaaggcactttatgatactttttctgcttttggaaacatactgtcctgcaaggtggtgtgtgatgagaacggctctaagggttatgcctttgtccacttcgagacccaagaggctgccgacaaggccatcgagaagatgaatggcatgctcctcaatgaccgcaaagtatttgtgggcagattcaagtctcgcaaagagcgggaagctgagcttggagccaaagccaaggaattcaccaatgtttatatcaaaaactttggggaagaggtggatgatgagagtctgaaagagctattcagtcagtttggtaagaccctaagtgtcaaggtgatgagagatcccaatgggaaatccaaaggctttggctttgtgagttacgaaaaacacgaggatgccaataaggctgtggaagagatgaatggaaaagaaataagtggtaaaatcatatttgtaggccgtgcacaaaagaaagtagaacggcaggcagagttaaaacggaaatttgaacagttgaaacaggagagaattagtcgatatcagggggtgaatctctacattaagaacttggatgacactattgatgatgagaaattaaggaaagaattttctccttttggatcaattaccagtgctaaggtaatgctggaggatggaagaagcaaagggtttggcttcgtctgcttctcatctcctgaagaagcaaccaaagcagtcactgagatgaatggacgcattgtgggctccaagccactatatgttgccctggcccagaggaaggaagagagaaaggctcacctgaccaaccagtatatgcaacgagtggctggaatgagagcacttcctgccaatgccatcttaaatcagttccagcctgcagcgggtggctactttgtgccagcagtcccacaggctcagggaaggcctccatattatacacctaaccagttagcacagatgaggcctaatccacgctggcagcaaggtgggagacctcaaggcttccaaggaatgccaagtgctatacgccagtctgggcctcgtccaactcttcgccatctggctccaactgggtctgagtgcccggaccgcttggctatggactttggtggggctggtgccgcccagcaagggctgactgacagctgccagtctggaggcgttcccacagctgtgcagaacttagcgccacgcgctgctgttgctgctgctgctccccgggctgttgccccctacaaatacgcctccagtgtccgcagccctcatcctgccatacagcctctgcaggcaccccagcctgcggtccatgtgcaggggcaggagccactgactgcctccatgctggctgcagcacccccccaggaacagaagcagatgctgggagaacgcttgttcccactcatccaaacaatgcattcaaatctggctgggaagatcacgggaatgctgctggagatagacaactctgagctgctgcacatgttagagtcccccgagtctctccgctccaaggtggatgaagctgtagcagttctacaggctcatcatgccaagaaagaagctgcccagaaggtgggcgctgttgctgctgctacctcttag

SEQ ID NO: 3 - DNA, 387 bp, Artificial Sequence
  MS2 (N55K)  - RNA binding protein fragment
gcttcaaactttactcagttcgtgctcgtggacaatggtgggacaggggatgtgacagtggctccttctaatttcgctaatggggtggcagagtggatcagctccaactcacggagccaggcctacaaggtgacatgcagcgtcaggcagtctagtgcccagaagagaaagtataccatcaaggtggaggtccccaaagtggctacccagacagtgggcggagtcgaactgcctgtcgccgcttggaggtcctacctgaacatggagctcactatcccaattttcgctaccaattctgactgtgaactcatcgtgaaggcaatgcaggggctcctcaaagacggtaatcctatcccttccgccatcgccgctaactcaggtatctac

SEQ ID NO: 4 - DNA, 4137 bp, Artificial Sequence
  dCas9 -  - RNA binding protein fragment
atgagccccaagaagaagagaaaggtggaggccagcgacaagaagtacagcatcggcctggccatcggcaccaactctgtgggctgggccgtgatcaccgacgagtacaaggtgcccagcaagaaattcaaggtgctgggcaacaccgaccggcacagcatcaagaagaacctgatcggagccctgctgttcgacagcggcgaaacagccgaggccacccggctgaagagaaccgccagaagaagatacaccagacggaagaaccggatctgctatctgcaagagatcttcagcaacgagatggccaaggtggacgacagcttcttccacagactggaagagtccttcctggtggaagaggataagaagcacgagcggcaccccatcttcggcaacatcgtggacgaggtggcctaccacgagaagtaccccaccatctaccacctgagaaagaaactggtggacagcaccgacaaggccgacctgcggctgatctatctggccctggcccacatgatcaagttccggggccacttcctgatcgagggcgacctgaaccccgacaacagcgacgtggacaagctgttcatccagctggtgcagacctacaaccagctgttcgaggaaaaccccatcaacgccagcggcgtggacgccaaggccatcctgtctgccagactgagcaagagcagacggctggaaaatctgatcgcccagctgcccggcgagaagaagaatggcctgttcggcaacctgattgccctgagcctgggcctgacccccaacttcaagagcaacttcgacctggccgaggatgccaaactgcagctgagcaaggacacctacgacgacgacctggacaacctgctggcccagatcggcgaccagtacgccgacctgtttctggccgccaagaacctgtccgacgccatcctgctgagcgacatcctgagagtgaacaccgagatcaccaaggcccccctgagcgcctctatgatcaagagatacgacgagcaccaccaggacctgaccctgctgaaagctctcgtgcggcagcagctgcctgagaagtacaaagagattttcttcgaccagagcaagaacggctacgccggctacattgacggcggagccagccaggaagagttctacaagttcatcaagcccatcctggaaaagatggacggcaccgaggaactgctcgtgaagctgaacagagaggacctgctgcggaagcagcggaccttcgacaacggcagcatcccccaccagatccacctgggagagctgcacgccattctgcggcggcaggaagatttttacccattcctgaaggacaaccgggaaaagatcgagaagatcctgaccttccgcatcccctactacgtgggccctctggccaggggaaacagcagattcgcctggatgaccagaaagagcgaggaaaccatcaccccctggaacttcgaggaagtggtggacaagggcgcttccgcccagagcttcatcgagcggatgaccaacttcgataagaacctgcccaacgagaaggtgctgcccaagcacagcctgctgtacgagtacttcaccgtgtataacgagctgaccaaagtgaaatacgtgaccgagggaatgagaaagcccgccttcctgagcggcgagcagaaaaaggccatcgtggacctgctgttcaagaccaaccggaaagtgaccgtgaagcagctgaaagaggactacttcaagaaaatcgagtgcttcgactccgtggaaatctccggcgtggaagatcggttcaacgcctccctgggcacataccacgatctgctgaaaattatcaaggacaaggacttcctggacaatgaggaaaacgaggacattctggaagatatcgtgctgaccctgacactgtttgaggacagagagatgatcgaggaacggctgaaaacctatgcccacctgttcgacgacaaagtgatgaagcagctgaagcggcggagatacaccggctggggcaggctgagccggaagctgatcaacggcatccgggacaagcagtccggcaagacaatcctggatttcctgaagtccgacggcttcgccaacagaaacttcatgcagctgatccacgacgacagcctgacctttaaagaggacatccagaaagcccaggtgtccggccagggcgatagcctgcacgagcacattgccaatctggccggcagccccgccattaagaagggcatcctgcagacagtgaaggtggtggacgagctcgtgaaagtgatgggccggcacaagcccgagaacatcgtgatcgaaatggccagagagaaccagaccacccagaagggacagaagaacagccgcgagagaatgaagcggatcgaagagggcatcaaagagctgggcagccagatcctgaaagaacaccccgtggaaaacacccagctgcagaacgagaagctgtacctgtactacctgcagaatgggcgggatatgtacgtggaccaggaactggacatcaaccggctgtccgactacgatgtggacgctatcgtgcctcagagctttctgaaggacgactccatcgacaacaaggtgctgaccagaagcgacaagaaccggggcaagagcgacaacgtgccctccgaagaggtcgtgaagaagatgaagaactactggcggcagctgctgaacgccaagctgattacccagagaaagttcgacaatctgaccaaggccgagagaggcggcctgagcgaactggataaggccggcttcatcaagagacagctggtggaaacccggcagatcacaaagcacgtggcacagatcctggactcccggatgaacactaagtacgacgagaatgacaagctgatccgggaagtgaaagtgatcaccctgaagtccaagctggtgtccgatttccggaaggatttccagttttacaaagtgcgcgagatcaacaactaccaccacgcccacgacgcctacctgaacgccgtcgtgggaaccgccctgatcaaaaagtaccctaagctggaaagcgagttcgtgtacggcgactacaaggtgtacgacgtgcggaagatgatcgccaagagcgagcaggaaatcggcaaggctaccgccaagtacttcttctacagcaacatcatgaactttttcaagaccgagattaccctggccaacggcgagatccggaagcggcctctgatcgagacaaacggcgaaaccggggagatcgtgtgggataagggccgggattttgccaccgtgcggaaagtgctgagcatgccccaagtgaatatcgtgaaaaagaccgaggtgcagacaggcggcttcagcaaagagtctatcctgcccaagaggaacagcgataagctgatcgccagaaagaaggactgggaccctaagaagtacggcggcttcgacagccccaccgtggcctattctgtgctggtggtggccaaagtggaaaagggcaagtccaagaaactgaagagtgtgaaagagctgctggggatcaccatcatggaaagaagcagcttcgagaagaatcccatcgactttctggaagccaagggctacaaagaagtgaaaaaggacctgatcatcaagctgcctaagtactccctgttcgagctggaaaacggccggaagagaatgctggcctctgccggcgaactgcagaagggaaacgaactggccctgccctccaaatatgtgaacttcctgtacctggccagccactatgagaagctgaagggctcccccgaggataatgagcagaaacagctgtttgtggaacagcacaagcactacctggacgagatcatcgagcagatcagcgagttctccaagagagtgatcctggccgacgctaatctggacaaagtgctgtccgcctacaacaagcaccgggataagcccatcagagagcaggccgagaatatcatccacctgtttaccctgaccaatctgggagcccctgccgccttcaagtactttgacaccaccatcgaccggaagaggtacaccagcaccaaagaggtgctggacgccaccctgatccaccagagcatcaccggcctgtacgagacacggatcgacctgtctcagctgggaggcgac

SEQ ID NO: 5 - DNA, 66 bp, Artificial Sequence
  p2A protein domain
ggatccggcgcaacaaacttctctctgctgaaacaagccggagatgtcgaagagaatcctggaccg

SEQ ID NO: 6 - DNA, 711 bp, Artificial Sequence
  YFP  protein domain
agcaagggcgaggagctgttcaccggggtggtgcccatcctggtcgagctggacggcgacgtaaacggccacaagttcagcgtgtccggcgagggcgagggcgatgccacctacggcaagctgaccctgaagttcatctgcaccaccggcaagctgcccgtgccctggcccaccctcgtgaccaccttcggctacggcctgcagtgcttcgcccgctaccccgaccacatgaagcagcacgacttcttcaagtccgccatgcccgaaggctacgtccaggagcgcaccatcttcttcaaggacgacggcaactacaagacccgcgccgaggtgaagttcgagggcgacaccctggtgaaccgcatcgagctgaagggcatcgacttcaaggaggacggcaacatcctggggcacaagctggagtacaactacaacagccacaacgtctatatcatggccgacaagcagaagaacggcatcaaggtgaacttcaagatccgccacaacatcgaggacggcagcgtgcagctcgccgaccactaccagcagaacacccccatcggcgacggccccgtgctgctgcccgacaaccactacctgagctaccagtccgccctgagcaaagaccccaacgagaagcgcgatcacatggtcctgctggagttcgtgaccgccgccgggatcactctcggcatggacgagctgtacaag

SEQ ID NO: 7 - DNA, 21 bp, Artificial Sequence
  GS6 linker
ggatcaggatcaggatcagga

SEQ ID NO: 8 - DNA, 204 bp, Artificial Sequence
  bGH pA terminator
cgactgtgccttctagttgccagccatctgttgtttgcccctcccccgtgccttccttgaccctggaaggtgccactcccactgtcctttcctaataaaatgaggaaattgcatcgcattgtctgagtaggtgtcattctattctggggggtggggtggggcaggacagcaagggggaggattgggaagacaatagcaggcatg

SEQ ID NO: 9 - DNA, 20 bp, Artificial Sequence
  spacer
ctgcaggtcgactctagaaa

SEQ ID NO: 10 - DNA, 19 bp, Artificial Sequence
  MS2 hairpin
acatgaggatcacccatgt

SEQ ID NO: 11 - DNA, 25 bp, Artificial Sequence
  Smartseq2 handle
aagcagtggtatcaacgcagagtac

SEQ ID NO: 12 - DNA, 24 bp, Artificial Sequence
  polyA capture
ttgttgttgttgttgttgtttttt